European Patent Specification EP 3 660 154 B1, published April 16, 2025. Title: Antisense Nucleic Acid. Applicant: NIPPON SHINYAKU CO., LTD. NATIONAL CENTER OF NEUROLOGY AND PSYCHIATRY. The sequence listing filed with the application follows.

SEQUENCE LISTING (128 sequences)

SEQ ID NO: 1 - DNA, 45 bp, Artificial
  Synthetic Nucleic Acid
ggcgatttgacagatctgttgagaaatggcggcgttttcattatg

SEQ ID NO: 2 - DNA, 58 bp, Artificial
  Synthetic Nucleic Acid
taatcagtggctaacagaagctgaacagtttctcagaaagacacaaattcctgagaat

SEQ ID NO: 3 - DNA, 17 bp, Artificial
  Synthetic Nucleic Acid
ttgagaaatggcggcgt

SEQ ID NO: 4 - DNA, 17 bp, Artificial
  Synthetic Nucleic Acid
tcagtggctaacagaag

SEQ ID NO: 5 - DNA, 17 bp, Artificial
  Synthetic Nucleic Acid
tctcagaaagacacaaa

SEQ ID NO: 6 - DNA, 26 bp, Artificial
  Synthetic Nucleic Acid
gtgtctttctgagccgccatttctca

SEQ ID NO: 7 - DNA, 22 bp, Artificial
  Synthetic Nucleic Acid
tctgttagccacgccgccattt

SEQ ID NO: 8 - DNA, 24 bp, Artificial
  Synthetic Nucleic Acid
ctgttagccactcgccgccatttc

SEQ ID NO: 9 - DNA, 24 bp, Artificial
  Synthetic Nucleic Acid
ttgtgtctttcttctgttagccac

SEQ ID NO: 10 - DNA, 148 bp, Homo sapiens
gcgatttgacagatctgttgagaaatggcggcgttttcattatgatataaagatatttaatcagtggctaacagaagctgaacagtttctcagaaagacacaaattcctgagaattgggaacatgctaaatacaaatggtatcttaag

SEQ ID NO: 11 - DNA, 26 bp, Artificial
  Synthetic Nucleic Acid
ttgtgtctttctgtctcaacagatct

SEQ ID NO: 12 - DNA, 26 bp, Artificial
  Synthetic Nucleic Acid
tgttagccactgatctcaacagatct

SEQ ID NO: 13 - DNA, 26 bp, Artificial
  Synthetic Nucleic Acid
gttcagcttctgttctcaacagatct

SEQ ID NO: 14 - DNA, 26 bp, Artificial
  Synthetic Nucleic Acid
ttgtgtctttctgcgccgccatttct

SEQ ID NO: 15 - DNA, 26 bp, Artificial
  Synthetic Nucleic Acid
ctgagaaactgttcgccgccatttct

SEQ ID NO: 16 - DNA, 26 bp, Artificial
  Synthetic Nucleic Acid
tctcaggaatttgcgccgccatttct

SEQ ID NO: 17 - DNA, 26 bp, Artificial
  Synthetic Nucleic Acid
tgttagccactgacgccgccatttct

SEQ ID NO: 18 - DNA, 26 bp, Artificial
  Synthetic Nucleic Acid
gttcagcttctgtcgccgccatttct

SEQ ID NO: 19 - DNA, 30 bp, Artificial
  Synthetic Nucleic Acid
attctcaggaatttgaacgccgccatttct

SEQ ID NO: 20 - DNA, 30 bp, Artificial
  Synthetic Nucleic Acid
atttgtgtctttctgtttctcaacagatct

SEQ ID NO: 21 - DNA, 25 bp, Artificial
  Synthetic Nucleic Acid
attctcaggaatttgtttctcaaca

SEQ ID NO: 22 - DNA, 30 bp, Artificial
  Synthetic Nucleic Acid
atttgtgtctttctgaacgccgccatttct

SEQ ID NO: 23 - DNA, 26 bp, Artificial
  Synthetic Nucleic Acid
tctcaggaatttgtctcaacagatct

SEQ ID NO: 24 - DNA, 26 bp, Artificial
  Synthetic Nucleic Acid
ttgtgtctttctgaacgccgccattt

SEQ ID NO: 25 - DNA, 26 bp, Artificial
  Synthetic Nucleic Acid
ttgtgtctttctgccgccatttctca

SEQ ID NO: 26 - DNA, 26 bp, Artificial
  Synthetic Nucleic Acid
gtgtctttctgagcgccgccatttct

SEQ ID NO: 27 - DNA, 26 bp, Artificial
  Synthetic Nucleic Acid
ctgagaaactgtttctcaacagatct

SEQ ID NO: 28 - DNA, 26 bp, Artificial
  Synthetic Nucleic Acid
atttgtgtctttcccgccatttctca

SEQ ID NO: 29 - DNA, 26 bp, Artificial
  Synthetic Nucleic Acid
gtgtctttctgagaacgccgccattt

SEQ ID NO: 30 - DNA, 26 bp, Artificial
  Synthetic Nucleic Acid
atttgtgtctttcaacgccgccattt

SEQ ID NO: 31 - DNA, 24 bp, Artificial
  Synthetic Nucleic Acid
ttgtgtctttctcgccgccatttc

SEQ ID NO: 32 - DNA, 26 bp, Artificial
  Synthetic Nucleic Acid
cgccgccatttctttgtgtctttctg

SEQ ID NO: 33 - DNA, 22 bp, Artificial
  Synthetic Nucleic Acid
tgtgtctttctgccgccatttc

SEQ ID NO: 34 - DNA, 20 bp, Artificial
  Synthetic Nucleic Acid
tgtgtctttcccgccatttc

SEQ ID NO: 35 - DNA, 26 bp, Artificial
  Synthetic Nucleic Acid
ttagccactgattccgccatttctca

SEQ ID NO: 36 - DNA, 26 bp, Artificial
  Synthetic Nucleic Acid
atttgtgtctttccgccgccatttct

SEQ ID NO: 37 - DNA, 26 bp, Artificial
  Synthetic Nucleic Acid
tctgttagccactcgccgccatttct

SEQ ID NO: 38 - DNA, 26 bp, Artificial
  Synthetic Nucleic Acid
tgttagccactgaccgccatttctca

SEQ ID NO: 39 - DNA, 26 bp, Artificial
  Synthetic Nucleic Acid
tctgttagccactccgccatttctca

SEQ ID NO: 40 - DNA, 26 bp, Artificial
  Synthetic Nucleic Acid
ttagccactgattcgccgccatttct

SEQ ID NO: 41 - DNA, 26 bp, Artificial
  Synthetic Nucleic Acid
tgttagccactgaaacgccgccattt

SEQ ID NO: 42 - DNA, 26 bp, Artificial
  Synthetic Nucleic Acid
tctgttagccactaacgccgccattt

SEQ ID NO: 43 - DNA, 26 bp, Artificial
  Synthetic Nucleic Acid
ttagccactgattaacgccgccattt

SEQ ID NO: 44 - DNA, 26 bp, Artificial
  Synthetic Nucleic Acid
ttgtgtctttctgtgttagccactga

SEQ ID NO: 45 - DNA, 26 bp, Artificial
  Synthetic Nucleic Acid
tgttcagcttctgtgttagccactga

SEQ ID NO: 46 - DNA, 20 bp, Artificial
  Synthetic Nucleic Acid
ttagccactgcgccgccatt

SEQ ID NO: 47 - DNA, 20 bp, Artificial
  Synthetic Nucleic Acid
ctgttagccacgccgccatt

SEQ ID NO: 48 - DNA, 20 bp, Artificial
  Synthetic Nucleic Acid
tgttcagctttagccactga

SEQ ID NO: 49 - DNA, 20 bp, Artificial
  Synthetic Nucleic Acid
ctgttagccaccgccatttc

SEQ ID NO: 50 - DNA, 26 bp, Artificial
  Synthetic Nucleic Acid
ttgtgtctttctggccatttctcaac

SEQ ID NO: 51 - DNA, 25 bp, Artificial
  Synthetic Nucleic Acid
ctgttagccactgcataatgaaaac

SEQ ID NO: 52 - DNA, 24 bp, Artificial
  Synthetic Nucleic Acid
ttctgttagccaaaaacgccgcca

SEQ ID NO: 53 - DNA, 22 bp, Artificial
  Synthetic Nucleic Acid
ttagccactgacgccgccattt

SEQ ID NO: 54 - DNA, 22 bp, Artificial
  Synthetic Nucleic Acid
ctgttagccacgccgccatttc

SEQ ID NO: 55 - DNA, 20 bp, Artificial
  Synthetic Nucleic Acid
actgttcagcgccactgatt

SEQ ID NO: 56 - DNA, 26 bp, Artificial
  Synthetic Nucleic Acid
aactgttcagctttagccactgatta

SEQ ID NO: 57 - DNA, 26 bp, Artificial
  Synthetic Nucleic Acid
ctgagaaactgtttgttagccactga

SEQ ID NO: 58 - DNA, 22 bp, Artificial
  Synthetic Nucleic Acid
aacgccgccatttgtgtctttc

SEQ ID NO: 59 - DNA, 28 bp, Artificial
  Synthetic Nucleic Acid
tgtgtctttctgttagccatttctcaac

SEQ ID NO: 60 - DNA, 24 bp, Artificial
  Synthetic Nucleic Acid
cgccgccatttcttgtgtctttct

SEQ ID NO: 61 - DNA, 26 bp, Artificial
  Synthetic Nucleic Acid
ccgccatttctcattgtgtctttctg

SEQ ID NO: 62 - DNA, 26 bp, Artificial
  Synthetic Nucleic Acid
ccgccatttctcatgttagccactga

SEQ ID NO: 63 - DNA, 26 bp, Artificial
  Synthetic Nucleic Acid
ctttctgagaaactgttagccactga

SEQ ID NO: 64 - DNA, 25 bp, Artificial
  Synthetic Nucleic Acid
gccactgacctctcagcttctgtta

SEQ ID NO: 65 - DNA, 26 bp, Artificial
  Synthetic Nucleic Acid
aacgccgccatttatttgtgtctttc

SEQ ID NO: 66 - DNA, 26 bp, Artificial
  Synthetic Nucleic Acid
aaacgccgccatttgtgtctttctga

SEQ ID NO: 67 - DNA, 20 bp, Artificial
  Synthetic Nucleic Acid
ctttctgttagccactgaac

SEQ ID NO: 68 - DNA, 26 bp, Artificial
  Synthetic Nucleic Acid
cgccgccatttcttttctgagaaact

SEQ ID NO: 69 - DNA, 26 bp, Artificial
  Synthetic Nucleic Acid
aacgccgccatttctgagaaactgtt

SEQ ID NO: 70 - DNA, 24 bp, Artificial
  Synthetic Nucleic Acid
cccagcttctgttagccactgacc

SEQ ID NO: 71 - DNA, 24 bp, Artificial
  Synthetic Nucleic Acid
cttgcttctgttagccactgaccc

SEQ ID NO: 72 - DNA, 21 bp, Artificial
  Synthetic Nucleic Acid
cgccgccatttctgagaaact

SEQ ID NO: 73 - DNA, 26 bp, Artificial
  Synthetic Nucleic Acid
ccgccatttctcagtgtctttctgag

SEQ ID NO: 74 - DNA, 26 bp, Artificial
  Synthetic Nucleic Acid
tgttagccactgattgtgtctttctg

SEQ ID NO: 75 - DNA, 26 bp, Artificial
  Synthetic Nucleic Acid
atttgtgtctttctgttagccactga

SEQ ID NO: 76 - DNA, 22 bp, Artificial
  Synthetic Nucleic Acid
gtctttctgagcgccatttctc

SEQ ID NO: 77 - DNA, 22 bp, Artificial
  Synthetic Nucleic Acid
ttgtgtctttcctgttagccac

SEQ ID NO: 78 - DNA, 24 bp, Artificial
  Synthetic Nucleic Acid
tgtctttctgagccgccatttctc

SEQ ID NO: 79 - DNA, 26 bp, Artificial
  Synthetic Nucleic Acid
aaactgttcagcttctgtcaaatcgc

SEQ ID NO: 80 - DNA, 26 bp, Artificial
  Synthetic Nucleic Acid
acgccgccatttctcaggaatttgtg

SEQ ID NO: 81 - DNA, 20 bp, Artificial
  Synthetic Nucleic Acid
ctgttcagctccactgatta

SEQ ID NO: 82 - DNA, 20 bp, Artificial
  Synthetic Nucleic Acid
actgttcagcccactgatta

SEQ ID NO: 83 - DNA, 22 bp, Artificial
  Synthetic Nucleic Acid
tgtgtctttctcgccgccattt

SEQ ID NO: 84 - DNA, 22 bp, Artificial
  Synthetic Nucleic Acid
tgtctttctgacgccatttctc

SEQ ID NO: 85 - DNA, 24 bp, Artificial
  Synthetic Nucleic Acid
cgccgccatttctttgtgtctttc

SEQ ID NO: 86 - DNA, 22 bp, Artificial
  Synthetic Nucleic Acid
cgccgccatttttgtgtctttc

SEQ ID NO: 87 - DNA, 20 bp, Artificial
  Synthetic Nucleic Acid
ctgttcagcttgttagccac

SEQ ID NO: 88 - DNA, 21 bp, Artificial
  Synthetic Nucleic Acid
ttctgagaaactgttagccac

SEQ ID NO: 89 - DNA, 18 bp, Artificial
  Synthetic Nucleic Acid
ctgttcagccactgatta

SEQ ID NO: 90 - DNA, 20 bp, Artificial
  Synthetic Nucleic Acid
ctgagaaacttgttagccac

SEQ ID NO: 91 - DNA, 22 bp, Artificial
  Synthetic Nucleic Acid
tgtctttctgaccgccatttct

SEQ ID NO: 92 - DNA, 22 bp, Artificial
  Synthetic Nucleic Acid
ctttctgagaacgccatttctc

SEQ ID NO: 93 - DNA, 19 bp, Artificial
  Synthetic Nucleic Acid
ctttctgagaaacgccgcc

SEQ ID NO: 94 - DNA, 23 bp, Artificial
  Synthetic Nucleic Acid
tgtctttctgttagccatttctc

SEQ ID NO: 95 - DNA, 20 bp, Artificial
  Synthetic Nucleic Acid
ctttctgttagccatttctc

SEQ ID NO: 96 - DNA, 20 bp, Artificial
  Synthetic Nucleic Acid
ctttctgagagccatttctc

SEQ ID NO: 97 - DNA, 22 bp, Artificial
  Synthetic Nucleic Acid
ctgttagccactccgccatttc

SEQ ID NO: 98 - DNA, 21 bp, Artificial
  Synthetic Nucleic Acid
ctgtgtctttctgttagccac

SEQ ID NO: 99 - DNA, 21 bp, Artificial
  Synthetic Nucleic Acid
ctgttcagcgccactgattac

SEQ ID NO: 100 - DNA, 24 bp, Artificial
  Synthetic Nucleic Acid
ctttctgagaaacgccgccatttc

SEQ ID NO: 101 - DNA, 25 bp, Artificial
  Synthetic Nucleic Acid
tgtctttctgagccgccatttctca

SEQ ID NO: 102 - DNA, 21 bp, Artificial
  Synthetic Nucleic Acid
ctttctgagaaccgccatttc

SEQ ID NO: 103 - DNA, 24 bp, Artificial
  Synthetic Nucleic Acid
tgttagccactgtgtcaaatcgcc

SEQ ID NO: 104 - DNA, 24 bp, Artificial
  Synthetic Nucleic Acid
tgtctttctgagtgtcaaatcgcc

SEQ ID NO: 105 - DNA, 24 bp, Artificial
  Synthetic Nucleic Acid
ccgccatttctctgtcaaatcgcc

SEQ ID NO: 106 - DNA, 25 bp, Artificial
  Synthetic Nucleic Acid
gtgtctttctgagccgccatttctc

SEQ ID NO: 107 - DNA, 25 bp, Artificial
  Synthetic Nucleic Acid
gtgtctttctgaccgccatttctca

SEQ ID NO: 108 - DNA, 24 bp, Artificial
  Synthetic Nucleic Acid
gtgtctttctgaccgccatttctc

SEQ ID NO: 109 - DNA, 21 bp, Artificial
  Synthetic Nucleic Acid
ttcagcttctgtcaaatcgcc

SEQ ID NO: 110 - DNA, 22 bp, Artificial
  Synthetic Nucleic Acid
tgttagccactgtcaaatcgcc

SEQ ID NO: 111 - DNA, 22 bp, Artificial
  Synthetic Nucleic Acid
tgtctttctgagtcaaatcgcc

SEQ ID NO: 112 - DNA, 22 bp, Artificial
  Synthetic Nucleic Acid
cgccatttctcgtcaaatcgcc

SEQ ID NO: 113 - DNA, 23 bp, Artificial
  Synthetic Nucleic Acid
gtgtctttctgccgccatttctc

SEQ ID NO: 114 - DNA, 12 bp, Artificial
  Synthetic Nucleic Acid
ccgccatttctc

SEQ ID NO: 115 - DNA, 11 bp, Artificial
  Synthetic Nucleic Acid
tctgttagcca

SEQ ID NO: 116 - DNA, 11 bp, Artificial
  Synthetic Nucleic Acid
cgccgccattt

SEQ ID NO: 117 - DNA, 12 bp, Artificial
  Synthetic Nucleic Acid
ttgtgtctttct

SEQ ID NO: 118 - DNA, 12 bp, Artificial
  Synthetic Nucleic Acid
tctgttagccac

SEQ ID NO: 119 - DNA, 13 bp, Artificial
  Synthetic Nucleic Acid
gtgtctttctgag

SEQ ID NO: 120 - DNA, 13 bp, Artificial
  Synthetic Nucleic Acid
ccgccatttctca

SEQ ID NO: 121 - DNA, 12 bp, Artificial
  Synthetic Nucleic Acid
ctgttagccact

SEQ ID NO: 122 - DNA, 12 bp, Artificial
  Synthetic Nucleic Acid
cgccgccatttc

SEQ ID NO: 123 - DNA, 10 bp, Artificial
  Synthetic Nucleic Acid
gccactgatt

SEQ ID NO: 124 - DNA, 10 bp, Artificial
  Synthetic Nucleic Acid
actgttcagc

SEQ ID NO: 125 - DNA, 20 bp, Artificial
  Synthetic Nucleic Acid
gctcaggtcggattgacatt

SEQ ID NO: 126 - DNA, 20 bp, Artificial
  Synthetic Nucleic Acid
gggcaactcttccaccagta

SEQ ID NO: 127 - DNA, 963 bp, Homo sapiens
  CDS (1)..(963)
atggagctactgtcgccaccgctccgcgacgtagacctgacggcccccgacggctctctctgctcctttgccacaacggacgacttctatgacgacccgtgtttcgactccccggacctgcgcttcttcgaagacctggacccgcgcctgatgcacgtgggcgcgctcctgaaacccgaagagcactcgcacttccccgcggcggtgcacccggccccgggcgcacgtgaggacgagcatgtgcgcgcgcccagcgggcaccaccaggcgggccgctgcctactgtgggcctgcaaggcgtgcaagcgcaagaccaccaacgccgaccgccgcaaggccgccaccatgcgcgagcggcgccgcctgagcaaagtaaatgaggcctttgagacactcaagcgctgcacgtcgagcaatccaaaccagcggttgcccaaggtggagatcctgcgcaacgccatccgctatatcgagggcctgcaggctctgctgcgcgaccaggacgccgcgccccctggcgccgcagccgccttctatgcgccgggcccgctgcccccgggccgcggcggcgagcactacagcggcgactccgacgcgtccagcccgcgctccaactgctccgacggcatgatggactacagcggccccccgagcggcgcccggcggcggaactgctacgaaggcgcctactacaacgaggcgcccagcgaacccaggcccgggaagagtgcggcggtgtcgagcctagactgcctgtccagcatcgtggagcgcatctccaccgagagccctgcggcgcccgccctcctgctggcggacgtgccttctgagtcgcctccgcgcaggcaagaggctgccgcccccagcgagggagagagcagcggcgaccccacccagtcaccggacgccgccccgcagtgccctgcgggtgcgaaccccaacccgatataccaggtgctctga

SEQ ID NO: 128 - protein, 320 aa, Homo sapiens
MELLSPPLRDVDLTAPDGSLCSFATTDDFYDDPCFDSPDLRFFEDLDPRLMHVGALLKPEEHSHFPAAVHPAPGAREDEHVRAPSGHHQAGRCLLWACKACKRKTTNADRRKAATMRERRRLSKVNEAFETLKRCTSSNPNQRLPKVEILRNAIRYIEGLQALLRDQDAAPPGAAAAFYAPGPLPPGRGGEHYSGDSDASSPRSNCSDGMMDYSGPPSGARRRNCYEGAYYNEAPSEPRPGKSAAVSSLDCLSSIVERISTESPAAPALLLADVPSESPPRRQEAAAPSEGESSGDPTQSPDAAPQCPAGANPNPIYQVL